European Patent Application EP 4 703 473 A1, published March 4, 2026. Title: NON-METHYLATED CpG OLIGODEOXYNUCLEOTIDE AND APPLICATION THEREOF. Applicant: BEIJING RAY MEDICINE BIOTECHNOLOGY CO. The sequence listing filed with the application follows.

SEQUENCE LISTING (6 sequences)

SEQ ID NO: 1 - DNA, 20 bp, synthetic construct
  misc_feature 1..20: note = ODN-1826
  source 1..20: mol_type = other DNA
tccatgacgttcctgacgtt

SEQ ID NO: 2 - DNA, 20 bp, synthetic construct
  misc_feature 1..20: note = AODN
  source 1..20: mol_type = other DNA
ggggggtcaacgttgagggg

SEQ ID NO: 3 - DNA, 12 bp, synthetic construct
  misc_feature 1..12: note = ODN-4084
  source 1..12: mol_type = other DNA
cctggatgggaa

SEQ ID NO: 4 - DNA, 42 bp, synthetic construct
  misc_feature 1..42: note = ODN ACT-1
  source 1..42: mol_type = other DNA
tccatgacgttcctgacgttattccatgacgttcctgacgtt

SEQ ID NO: 5 - DNA, 42 bp, synthetic construct
  misc_feature 1..42: note = ODN ACT-2
  source 1..42: mol_type = other DNA
tccatgacgttcctgacgttcgtccatgacgttcctgacgtt

SEQ ID NO: 6 - DNA, 40 bp, synthetic construct
  misc_feature 1..40: note = ODN ACT-3
  source 1..40: mol_type = other DNA
tccatgacgttcctgacgttggggggtcaacgttgagggg